European Patent Application EP 4 534 661 A1, published April 9, 2025. Title: Mutant microorganism of Corynebacterium genus producing L-glutamic acid and method for producing L-glutamic acid using the same. Applicant: DAESANG CORPORATION. The sequence listing filed with the application follows.

SEQUENCE LISTING (9 sequences)

SEQ ID NO: 1 - DNA, 693 bp, synthetic construct
  source 1..693: mol_type = other DNA
atgaatcctataaccgaattattagacgcaacattatggatcggcggagttccgattctgtggcgcgaaatcatcggcaacgttttcggattatttagcgcgtgggcaggaatgcgacgcatcgtgtgggcatggcccatcggcatcataggcaacgcgctgctgttcacagtatttatgggcggccttttccacactccacaaaacctcgatctctacggccaagcgggtcgccagatcatgttcatcatcgtcagtggttatggctggtaccaatggtcggccgcaaaacgtcgcgcactcaccccagaaaatgcagtagcagtggttcctcgctgggcaagcaccaaagaacgcgccggcattgtgatcgcagcggttgtcggaacactcagcttcgcctggattttccaagcacttggctcctggggaccatgggccgacgcgtggattttcgtcggctcaatcctggctacctacggaatgactcgcggatggacagagttctggctgatctggatcgccgtcgacatagttggcgttcctctacttttgactgctggctactacccatccgcggtgctttacctggtgtatggcgcgtttgtcagctggggatttgtcgtgtggctgcgggtgcaaaaagcagacaaggctcgtgcgctggaagctcaagagtctgtgacagtctga

SEQ ID NO: 2 - protein, 230 aa, synthetic construct
MNPITELLDATLWIGGVPILWREIIGNVFGLFSAWAGMRRIVWAWPIGIIGNALLFTVFMGGLFHTPQNLDLYGQAGRQIMFIIVSGYGWYQWSAAKRRALTPENAVAVVPRWASTKERAGIVIAAVVGTLSFAWIFQALGSWGPWADAWIFVGSILATYGMTRGWTEFWLIWIAVDIVGVPLLLTAGYYPSAVLYLVYGAFVSWGFVVWLRVQKADKARALEAQESVTV

SEQ ID NO: 3 - DNA, 693 bp, Corynebacterium sp.
  source 1..693: mol_type = genomic DNA
atgaatcctataaccgaattattagacgcaacattatggatcggcggagttccgattctgtggcgcgaaatcatcggcaacgttttcggattatttagcgcgtgggcaggaatgcgacgcatcgtgtgggcatggcccatcggcatcataggcaacgcgctgctgttcacagtatttatgggcggccttttccacactccacaaaacctcgatctctacggccaagcgggtcgccagatcatgttcatcatcgtcagtggttatggctggtaccaatggtcggccgcaaaacgtcgcgcactcaccccagaaaatgcagtagcagtggttcctcgctgggcaagcaccaaagaacgcgccggcattgtgatcgcagcggttgtcggaacactcagcttcgcctggattttccaagcacttggctcctggggaccatgggccgacgcgtggattttcgtcggctcaatcctggctacctacggaatggctcgcggatggacagagttctggctgatctggatcgccgtcgacatagttggcgttcctctacttttgactgctggctactacccatccgcggtgctttacctggtgtatggcgcgtttgtcagctggggatttgtcgtgtggctgcgggtgcaaaaagcagacaaggctcgtgcgctggaagctcaagagtctgtgacagtctga

SEQ ID NO: 4 - protein, 230 aa, Corynebacterium sp.
MNPITELLDATLWIGGVPILWREIIGNVFGLFSAWAGMRRIVWAWPIGIIGNALLFTVFMGGLFHTPQNLDLYGQAGRQIMFIIVSGYGWYQWSAAKRRALTPENAVAVVPRWASTKERAGIVIAAVVGTLSFAWIFQALGSWGPWADAWIFVGSILATYGMARGWTEFWLIWIAVDIVGVPLLLTAGYYPSAVLYLVYGAFVSWGFVVWLRVQKADKARALEAQESVTV

SEQ ID NO: 5 - DNA, 5719 bp, synthetic construct
  source 1..5719: mol_type = other DNA
tgccgcaagcactcagggcgcaagggctgctaaaggaagcggaacacgtagaaagccagtccgcagaaacggtgctgaccccggatgaatgtcagctactgggctatctggacaagggaaaacgcaagcgcaaagagaaagcaggtagcttgcagtgggcttacatggcgatagctagactgggcggttttatggacagcaagcgaaccggaattgccagctggggcgccctctggtaaggttgggaagccctgcaaagtaaactggatggctttcttgccgccaaggatctgatggcgcaggggatcaagatctgatcaagagacaggatgaggatcgtttcgcatgattgaacaagatggattgcacgcaggttctccggccgcttgggtggagaggctattcggctatgactgggcacaacagacaatcggctgctctgatgccgccgtgttccggctgtcagcgcaggggcgcccggttctttttgtcaagaccgacctgtccggtgccctgaatgaactccaagacgaggcagcgcggctatcgtggctggccacgacgggcgttccttgcgcagctgtgctcgacgttgtcactgaagcgggaagggactggctgctattgggcgaagtgccggggcaggatctcctgtcatctcaccttgctcctgccgagaaagtatccatcatggctgatgcaatgcggcggctgcatacgcttgatccggctacctgcccattcgaccaccaagcgaaacatcgcatcgagcgagcacgtactcggatggaagccggtcttgtcgatcaggatgatctggacgaagagcatcaggggctcgcgccagccgaactgttcgccaggctcaaggcgcggatgcccgacggcgaggatctcgtcgtgacccatggcgatgcctgcttgccgaatatcatggtggaaaatggccgcttttctggattcatcgactgtggccggctgggtgtggcggaccgctatcaggacatagcgttggctacccgtgatattgctgaagagcttggcggcgaatgggctgaccgcttcctcgtgctttacggtatcgccgctcccgattcgcagcgcatcgccttctatcgccttcttgacgagttcttctgagcgggactctggggttcgctagaggatcgatcctttttaacccatcacatatacctgccgttcactattatttagtgaaatgagatattatgatattttctgaattgtgattaaaaaggcaactttatgcccatgcaacagaaactataaaaaatacagagaatgaaaagaaacagatagattttttagttctttaggcccgtagtctgcaaatccttttatgattttctatcaaacaaaagaggaaaatagaccagttgcaatccaaacgagagtctaatagaatgaggtcgaaaagtaaatcgcgcgggtttgttactgataaagcaggcaagacctaaaatgtgtaaagggcaaagtgtatactttggcgtcaccccttacatattttaggtctttttttattgtgcgtaactaacttgccatcttcaaacaggagggctggaagaagcagaccgctaacacagtacataaaaaaggagacatgaacgatgaacatcaaaaagtttgcaaaacaagcaacagtattaacctttactaccgcactgctggcaggaggcgcaactcaagcgtttgcgaaagaaacgaaccaaaagccatataaggaaacatacggcatttcccatattacacgccatgatatgctgcaaatccctgaacagcaaaaaaatgaaaaatatcaagtttctgaatttgattcgtccacaattaaaaatatctcttctgcaaaaggcctggacgtttgggacagctggccattacaaaacgctgacggcactgtcgcaaactatcacggctaccacatcgtctttgcattagccggagatcctaaaaatgcggatgacacatcgatttacatgttctatcaaaaagtcggcgaaacttctattgacagctggaaaaacgctggccgcgtctttaaagacagcgacaaattcgatgcaaatgattctatcctaaaagaccaaacacaagaatggtcaggttcagccacatttacatctgacggaaaaatccgtttattctacactgatttctccggtaaacattacggcaaacaaacactgacaactgcacaagttaacgtatcagcatcagacagctctttgaacatcaacggtgtagaggattataaatcaatctttgacggtgacggaaaaacgtatcaaaatgtacagcagttcatcgatgaaggcaactacagctcaggcgacaaccatacgctgagagatcctcactacgtagaagataaaggccacaaatacttagtatttgaagcaaacactggaactgaagatggctaccaaggcgaagaatctttatttaacaaagcatactatggcaaaagcacatcattcttccgtcaagaaagtcaaaaacttctgcaaagcgataaaaaacgcacggctgagttagcaaacggcgctctcggtatgattgagctaaacgatgattacacactgaaaaaagtgatgaaaccgctgattgcatctaacacagtaacagatgaaattgaacgcgcgaacgtctttaaaatgaacggcaaatggtacctgttcactgactcccgcggatcaaaaatgacgattgacggcattacgtctaacgatatttacatgcttggttatgtttctaattctttaactggcccatacaagccgctgaacaaaactggccttgtgttaaaaatggatcttgatcctaacgatgtaacctttacttactcacacttcgctgtacctcaagcgaaaggaaacaatgtcgtgattacaagctatatgacaaacagaggattctacgcagacaaacaatcaacgtttgcgccgagcttcctgctgaacatcaaaggcaagaaaacatctgttgtcaaagacagcatccttgaacaaggacaattaacagttaacaaataaaaacgcaaaagaaaatgccgatgggtaccgagcgaaatgaccgaccaagcgacgcccaacctgccatcacgagatttcgattccaccgccgccttctatgaaaggttgggcttcggaatcgttttccgggacgccctcgcggacgtgctcatagtccacgacgcccgtgattttgtagccctggccgacggccagcaggtaggccgacaggctcatgccggccgccgccgccttttcctcaatcgctcttcgttcgtctggaaggcagtacaccttgataggtgggctgcccttcctggttggcttggtttcatcagccatccgcttgccctcatctgttacgccggcggtagccggccagcctcgcagagcaggattcccgttgagcaccgccaggtgcgaataagggacagtgaagaaggaacacccgctcgcgggtgggcctacttcacctatcctgcccggctgacgccgttggatacaccaaggaaagtctacacgaaccctttggcaaaatcctgtatatcgtgcgaaaaaggatggatataccgaaaaaatcgctataatgaccccgaagcagggttatgcagcggaaaagcgctgcttccctgctgttttgtggaatatctaccgactggaaacaggcaaatgcaggaaattactgaactgaggggacaggcgagagacgatgccaaagagctcctgaaaatctcgataactcaaaaaatacgcccggtagtgatcttatttcattatggtgaaagttggaacctcttacgtgccgatcaacgtctcattttcgccaaaagttggcccagggcttcccggtatcaacagggacaccaggatttatttattctgcgaagtgatcttccgtcacaggtatttattcggcgcaaagtgcgtcgggtgatgctgccaacttactgatttagtgtatgatggtgtttttgaggtgctccagtggcttctgtttctatcagctcctgaaaatctcgataactcaaaaaatacgcccggtagtgatcttatttcattatggtgaaagttggaacctcttacgtgccgatcaacgtctcattttcgccaaaagttggcccagggcttcccggtatcaacagggacaccaggatttatttattctgcgaagtgatcttccgtcacaggtatttattcggcgcaaagtgcgtcgggtgatgctgccaacttactgatttagtgtatgatggtgtttttgaggtgctccagtggcttctgtttctatcagggctggatgatcctccagcgcggggatctcatgctggagttcttcgcccaccccaaaaggatctaggtgaagatcctttttgataatctcatgaccaaaatcccttaacgtgagttttcgttccactgagcgtcagaccccgtagaaaagatcaaaggatcttcttgagatcctttttttctgcgcgtaatctgctgcttgcaaacaaaaaaaccaccgctaccagcggtggtttgtttgccggatcaagagctaccaactctttttccgaaggtaactggcttcagcagagcgcagataccaaatactgttcttctagtgtagccgtagttaggccaccacttcaagaactctgtagcaccgcctacatacctcgctctgctaatcctgttaccagtggctgctgccagtggcgataagtcgtgtcttaccgggttggactcaagacgatagttaccggataaggcgcagcggtcgggctgaacggggggttcgtgcacacagcccagcttggagcgaacgacctacaccgaactgagatacctacagcgtgagctatgagaaagcgccacgcttcccgaagggagaaaggcggacaggtatccggtaagcggcagggtcggaacaggagagcgcacgagggagcttccagggggaaacgcctggtatctttatagtcctgtcgggtttcgccacctctgacttgagcgtcgatttttgtgatgctcgtcaggggggcggagcctatggaaaaacgccagcaacgcggcctttttacggttcctggccttttgctggccttttgctcacatgttctttcctgcgttatcccctgattctgtggataaccgtattaccgcctttgagtgagctgataccgctcgccgcagccgaacgaccgagcgcagcgagtcagtgagcgaggaagcggaagagcgcccaatacgcaaaccgcctctccccgcgcgttggccgattcattaatgcagctggcacgacaggtttcccgactggaaagcgggcagtgagcgcaacgcaattaatgtgagttagctcactcattaggcaccccaggctttacactttatgcttccggctcgtatgttgtgtggaattgtgagcggataacaatttcacacaggaaacagctatgacatgattacgccaagcttgcatgcctgcaggtcgactctagaggatccccgggtaccgagctcgaattcactggccgtcgttttacaacgtcgtgactgggaaaaccctggcgttacccaacttaatcgccttgcagcacatccccctttcgccagctggcgtaatagcgaagaggcccgcaccgatcgcccttcccaacagttgcgcagcctgaatggcgaatggcgataagctagcttcacgc

SEQ ID NO: 6 - DNA, 23 bp, synthetic construct
  source 1..23: mol_type = other DNA
cagtttcaaccagggcggttcat

SEQ ID NO: 7 - DNA, 22 bp, synthetic construct
  source 1..22: mol_type = other DNA
catccgcgagtcattccgtagg

SEQ ID NO: 8 - DNA, 22 bp, synthetic construct
  source 1..22: mol_type = other DNA
cctacggaatgactcgcggatg

SEQ ID NO: 9 - DNA, 19 bp, synthetic construct
  source 1..19: mol_type = other DNA
gcctcgcccaagggtgtga